European Patent Application EP 4 458 842 A1, published November 6, 2024. Title: MUTANT OF ADENO-ASSOCIATED VIRUS CAPSID PROTEIN. Applicant: Industry-Academic Cooperation Foundation, Yonsei University. Application KR. The sequence listing filed with the application follows.

SEQUENCE LISTING (12 sequences)

SEQ ID NO: 1 - protein, 736 aa, Artificial Sequence
MAADGYLPDWLEDNLSEGIREWWDLKPGAPKPKANQQKQDDGRGLVLPGYKYLGPFNGLDKGEPVNAADAAALEHDKAYDQQLKAGDNPYLRYNHADAEFQERLQEDTSFGGNLGRAVFQAKKRVLEPLGLVEEGAKTAPGKKRPVEQSPQEPDSSSGIGKTGQQPAKKRLNFGQTGDSESVPDPQPLGEPPATPAAVGPTTMASGGGAPMADNNEGADGVGNASGNWHCDSTWLGDRVITTSTRTWALPTYNNHLYKQISSASTGASNDNHYFGYSTPWGYFDFNRFHCHFSPRDWQRLINNNWGFRPKRLNFKLFNIQVKEVTTNDGVTTIANNLTSTVQVFSDSEYQLPYVLGSAHQGCLPPFPADVFMIPQYGYLTLNNGSQAVGRSSFYCLEYFPSQMLRTGNNFTFSYTFEEVPFHSSYAHSQSLDRLMNPLIDQYLYYLNRTQNQSGSAQNKDLLFSRGSPAGMSVQPKNWLPGPCYRQQRVSKTKTDNNNSNFTWTGASKYNLNGRESIINPGTAMASHKDDEDKFFPMSGVMIFGKESAGASNTALDNVMITDEEEIKATNPVATERFGTVAVNFQSSSTDPATGDVHAMGALPGMVWQDRDVYLQGPIWAKIPHTDGHFHPSPLMGGFGLKNPPPQILIKNTPVPANPPAEFSATKFASFITQYSTGQVSVEIEWELQKENSKRWNPEVQYTSNYAKSANVDFTVDNNGLYTEPRPIGTRYLTRPL

SEQ ID NO: 2 - DNA, 2211 bp, Artificial Sequence
  source 1..2211: mol_type = unassigned DNA
atggctgccgatggttatcttccagattggctcgaggacaacctctctgagggcattcgcgagtggtgggacttgaaacctggagccccgaagcccaaagccaaccagcaaaagcaggacgacggccggggtctggtgcttcctggctacaagtacctcggacccttcaacggactcgacaagggggagcccgtcaacgcggcggacgcagcggccctcgagcacgacaaggcctacgaccagcagctcaaagcgggtgacaatccgtaccttcggtataaccacgccgacgccgagtttcaggagcgtctgcaagaagatacgtcttttgggggcaacctcgggcgagcagtcttccaggccaagaagcgggttctcgaacctctcggtctggttgaggaaggcgctaagacggctcctggaaagaaacgtccggtagagcagtcgccacaagagccagactcctcctcgggcatcggcaagacaggccagcagcccgctaaaaagagactcaattttggtcagactggcgactcagagtcagtccccgacccacaacctctcggagaacctccagcaacccccgctgctgtgggacctactacaatggcttcaggcggtggcgcaccaatggcagacaataacgaaggcgccgacggagtgggtaatgcctcaggaaattggcattgcgattccacatggctgggcgacagagtcatcaccaccagcacccgcacctgggccttgcccacctacaataaccacctctacaagcaaatctccagtgcttcaacgggggccagcaacgacaaccactacttcggctacagcaccccctgggggtattttgatttcaacagattccactgccacttttcaccacgtgactggcagcgactcatcaacaacaattggggattccggcccaagagactcaacttcaaactcttcaacatccaagtcaaggaggtcacgacgaatgatggcgtcacaaccatcgctaataaccttaccagcacggttcaagtcttctcggactcggagtaccagcttccgtacgtcctcggctctgcgcaccagggctgcctccctccgttcccggcggacgtgttcatgattccgcaatacggctacctgacgctcaacaatggcagccaagccgtgggacgttcatccttttactgcctggaatatttcccttctcagatgctgagaacgggcaacaactttaccttcagctacacctttgaggaagtgcctttccacagcagctacgcgcacagccagagcctggaccggctgatgaatcctctcatcgaccaatacctgtattacctgaacagaactcaaaatcagtccggaagtgcccaaaacaaggacttgctgtttagccgtgggtctccagctggcatgtctgttcagcccaaaaactggctacctggaccctgttatcggcagcagcgcgtttctaaaacaaaaacagacaacaacaacagcaattttacctggactggtgcttcaaaatataacctcaatgggcgtgaatccatcatcaaccctggcactgctatggcctcacacaaagacgacgaagacaagttctttcccatgagcggtgtcatgatttttggaaaagagagcgccggagcttcaaacactgcattggacaatgtcatgattacagacgaagaggaaattaaagccactaaccctgtggccaccgaaagatttgggaccgtggcagtcaatttccagagcagcagcacagaccctgcgaccggagatgtgcatgctatgggagcattacctggcatggtgtggcaagatagagacgtgtacctgcagggtcccatttgggccaaaattccccacacagatggacactttcacccgtctcctcttatgggcggctttggactcaagaacccgcctcctcagatcctcatcaaaaacacgcctgttcctgcgaatcctccggcggagttttcagctacaaagtttgcttcattcatcacccaatactccacaggacaagtgagtgtggaaattgaatgggagctgcagaaagaaaacagcaagcgctggaatcccgaagtgcagtacacatccaattatgcaaaatctgccaacgttgattttactgtggacaacaatggactttatactgagcctcgccccattggcacccgttaccttacccgtcccctgtaa

SEQ ID NO: 3 - protein, 736 aa, Artificial Sequence
MAADGYLPDWLEDNLSEGIREWWDLKPGAPKPKANQQKQDDGRGLVLPGYKYLGPFNGLDKGEPVNAADAAALEHDKAYDQQLKAGDNPYLRYNHADAEFQERLQEDTSFGGNLGRAVFQAKKRVLEPLGLVEEGAKTAPGKKRPVEQSPQEPDSSSGIGKTGQQPAKKRLNFGQTGDSESVPDPQPLGEPPATPAAVGPTTMASGGGAPMADNNEGADGVGNASGNWHCDSTWLGDRVITTSTRTWALPTYNNHLYKQISSASTGASNDNHYFGYSTPWGYFDFNRFHCHFSPRDWQRLINNNWGFRPKRLNFKLFNIQVKEVTTNDGVTTIANNLTSTVQVFSDSEYQLPYVLGSAHQGCLPPFPADVFMIPQYGYLTLNNGSQAVGRSSFYCLEYFPSQMLRTGNNFTFSYTFEEVPFHSSYAHSQCLDRLMNPLIDQYLYYLNRTQNQSGSAQNKDLLFSRGSPAGMSVQPKNWLPGPCYRQQRVSKTKTDNNNSNFTWTGASKYNLNGRESIINPGTAMASHKDDEDKFFPMSGVMIFGKESAGASNTALDNVMITDEEEIKATNPVATERFGTVAVNFQSSSTDPATGDVHAMGALPGMVWQDRDVYLQGPIWAKIPHTDGHFHPSPLMGGFGLKNPPPQVLIKNTPVPANPPAEFSATKFASFITQYSTGQVSVEIEWELQKENSKRWNPEVQYTSNYAKSANVDFTVDNNGLYTEPRPIGTRYLTRPL

SEQ ID NO: 4 - DNA, 2211 bp, Artificial Sequence
  source 1..2211: mol_type = genomic DNA
atggctgccgatggttatcttccagattggctcgaggacaacctctctgagggcattcgcgagtggtgggacttgaaacctggagccccgaagcccaaagccaaccagcaaaagcaggacgacggccggggtctggtgcttcctggctacaagtacctcggacccttcaacggactcgacaagggggagcccgtcaacgcggcggacgcagcggccctcgagcacgacaaggcctacgaccagcagctcaaagcgggtgacaatccgtaccttcggtataaccacgccgacgccgagtttcaggagcgtctgcaagaagatacgtcttttgggggcaacctcgggcgagcagtcttccaggccaagaagcgggttctcgaacctctcggtctggttgaggaaggcgctaagacggctcctggaaagaaacgtccggtagagcagtcgccacaagagccagactcctcctcgggcatcggcaagacaggccagcagcccgctaaaaagagactcaattttggtcagactggcgactcagagtcagtccccgacccacaacctctcggagaacctccagcaacccccgctgctgtgggacctactacaatggcttcaggcggtggcgcaccaatggcagacaataacgaaggcgccgacggagtgggtaatgcctcaggaaattggcattgcgattccacatggctgggcgacagagtcatcaccaccagcacccgcacctgggccttgcccacctacaataaccacctctacaagcaaatctccagtgcttcaacgggggccagcaacgacaaccactacttcggctacagcaccccctgggggtattttgatttcaacagattccactgccacttttcaccacgtgactggcagcgactcatcaacaacaattggggattccggcccaagagactcaacttcaaactcttcaacatccaagtcaaggaggtcacgacgaatgatggcgtcacaaccatcgctaataaccttaccagcacggttcaagtcttctcggactcggagtaccagcttccgtacgtcctcggctctgcgcaccagggctgcctccctccgttcccggcggacgtgttcatgattccgcaatacggctacctgacgctcaacaatggcagccaagccgtgggacgttcatccttttactgcctggaatatttcccttctcagatgctgagaacgggcaacaactttaccttcagctacacctttgaggaagtgcctttccacagcagctacgcgcacagccagtgcctggaccggctgatgaatcctctcatcgaccaatacctgtattacctgaacagaactcaaaatcagtccggaagtgcccaaaacaaggacttgctgtttagccgtgggtctccagctggcatgtctgttcagcccaaaaactggctacctggaccctgttatcggcagcagcgcgtttctaaaacaaaaacagacaacaacaacagcaattttacctggactggtgcttcaaaatataacctcaatgggcgtgaatccatcatcaaccctggcactgctatggcctcacacaaagacgacgaagacaagttctttcccatgagcggtgtcatgatttttggaaaagagagcgccggagcttcaaacactgcattggacaatgtcatgattacagacgaagaggaaattaaagccactaaccctgtggccaccgaaagatttgggaccgtggcagtcaatttccagagcagcagcacagaccctgcgaccggagatgtgcatgctatgggagcattacctggcatggtgtggcaagatagagacgtgtacctgcagggtcccatttgggccaaaattccccacacagatggacactttcacccgtctcctcttatgggcggctttggactcaagaacccgcctcctcaggtcctcatcaaaaacacgcctgttcctgcgaatcctccggcggagttttcagctacaaagtttgcttcattcatcacccaatactccacaggacaagtgagtgtggaaattgaatgggagctgcagaaagaaaacagcaagcgctggaatcccgaagtgcagtacacatccaattatgcaaaatctgccaacgttgattttactgtggacaacaatggactttatactgagcctcgccccattggcacccgttaccttacccgtcccctgtaa

SEQ ID NO: 5 - DNA, 7328 bp, Artificial Sequence
  source 1..7328: mol_type = genomic DNA
gcgcgccgatatcgttaacgccccgcgccggccgctctagaactagtggatcccccggaagatcagaagttcctattccgaagttcctattctctagaaagtataggaacttctgatctgcgcagccgccatgccggggttttacgagattgtgattaaggtccccagcgaccttgacgggcatctgcccggcatttctgacagctttgtgaactgggtggccgagaaggaatgggagttgccgccagattctgacatggatctgaatctgattgagcaggcacccctgaccgtggccgagaagctgcagcgcgactttctgacggaatggcgccgtgtgagtaaggccccggaggcccttttctttgtgcaatttgagaagggagagagctacttccacatgcacgtgctcgtggaaaccaccggggtgaaatccatggttttgggacgtttcctgagtcagattcgcgaaaaactgattcagagaatttaccgcgggatcgagccgactttgccaaactggttcgcggtcacaaagaccagaaatggcgccggaggcgggaacaaggtggtggatgagtgctacatccccaattacttgctccccaaaacccagcctgagctccagtgggcgtggactaatatggaacagtatttaagcgcctgtttgaatctcacggagcgtaaacggttggtggcgcagcatctgacgcacgtgtcgcagacgcaggagcagaacaaagagaatcagaatcccaattctgatgcgccggtgatcagatcaaaaacttcagccaggtacatggagctggtcgggtggctcgtggacaaggggattacctcggagaagcagtggatccaggaggaccaggcctcatacatctccttcaatgcggcctccaactcgcggtcccaaatcaaggctgccttggacaatgcgggaaagattatgagcctgactaaaaccgcccccgactacctggtgggccagcagcccgtggaggacatttccagcaatcggatttataaaattttggaactaaacgggtacgatccccaatatgcggcttccgtctttctgggatgggccacgaaaaagttcggcaagaggaacaccatctggctgtttgggcctgcaactaccgggaagaccaacatcgcggaggccatagcccacactgtgcccttctacgggtgcgtaaactggaccaatgagaactttcccttcaacgactgtgtcgacaagatggtgatctggtgggaggaggggaagatgaccgccaaggtcgtggagtcggccaaagccattctcggaggaagcaaggtgcgcgtggaccagaaatgcaagtcctcggcccagatagacccgactcccgtgatcgtcacctccaacaccaacatgtgcgccgtgattgacgggaactcaacgaccttcgaacaccagcagccgttgcaagaccggatgttcaaatttgaactcacccgccgtctggatcatgactttgggaaggtcaccaagcaggaagtcaaagactttttccggtgggcaaaggatcacgtggttgaggtggagcatgaattctacgtcaaaaagggtggagccaagaaaagacccgcccccagtgacgcagatataagtgagcccaaacgggtgcgcgagtcagttgcgcagccatcgacgtcagacgcggaagcttcgatcaactacgcagacaggtaccaaaacaaatgttctcgtcacgtgggcatgaatctgatgctgtttccctgcagacaatgcgagagaatgaatcagaattcaaatatctgcttcactcacggacagaaagactgtttagagtgctttcccgtgtcagaatctcaacccgtttctgtcgtcaaaaaggcgtatcagaaactgtgctacattcatcatatcatgggaaaggtgccagacgcttgcactgcctgcgatctggtcaatgtggatttggatgactgcatctttgaacaataaatgatttaaatcaggtatggctgccgatggttatcttccagattggctcgaggacaacctctctgagggcattcgcgagtggtgggacttgaaacctggagccccgaagcccaaagccaaccagcaaaagcaggacgacggccggggtctggtgcttcctggctacaagtacctcggacccttcaacggactcgacaagggggagcccgtcaacgcggcggacgcagcggccctcgagcacgacaaggcctacgaccagcagctcaaagcgggtgacaatccgtaccttcggtataaccacgccgacgccgagtttcaggagcgtctgcaagaagatacgtcttttgggggcaacctcgggcgagcagtcttccaggccaagaagcgggttctcgaacctctcggtctggttgaggaaggcgctaagacggctcctggaaagaaacgtccggtagagcagtcgccacaagagccagactcctcctcgggcatcggcaagacaggccagcagcccgctaaaaagagactcaattttggtcagactggcgactcagagtcagtccccgacccacaacctctcggagaacctccagcaacccccgctgctgtgggacctactacaatggcttcaggcggtggcgcaccaatggcagacaataacgaaggcgccgacggagtgggtaatgcctcaggaaattggcattgcgattccacatggctgggcgacagagtcatcaccaccagcacccgcacctgggccttgcccacctacaataaccacctctacaagcaaatctccagtgcttcaacgggggccagcaacgacaaccactacttcggctacagcaccccctgggggtattttgatttcaacagattccactgccacttttcaccacgtgactggcagcgactcatcaacaacaattggggattccggcccaagagactcaacttcaaactcttcaacatccaagtcaaggaggtcacgacgaatgatggcgtcacaaccatcgctaataaccttaccagcacggttcaagtcttctcggactcggagtaccagcttccgtacgtcctcggctctgcgcaccagggctgcctccctccgttcccggcggacgtgttcatgattccgcaatacggctacctgacgctcaacaatggcagccaagccgtgggacgttcatccttttactgcctggaatatttcccttctcagatgctgagaacgggcaacaactttaccttcagctacacctttgaggaagtgcctttccacagcagctacgcgcacagccagtgcctggaccggctgatgaatcctctcatcgaccaatacctgtattacctgaacagaactcaaaatcagtccggaagtgcccaaaacaaggacttgctgtttagccgtgggtctccagctggcatgtctgttcagcccaaaaactggctacctggaccctgttatcggcagcagcgcgtttctaaaacaaaaacagacaacaacaacagcaattttacctggactggtgcttcaaaatataacctcaatgggcgtgaatccatcatcaaccctggcactgctatggcctcacacaaagacgacgaagacaagttctttcccatgagcggtgtcatgatttttggaaaagagagcgccggagcttcaaacactgcattggacaatgtcatgattacagacgaagaggaaattaaagccactaaccctgtggccaccgaaagatttgggaccgtggcagtcaatttccagagcagcagcacagaccctgcgaccggagatgtgcatgctatgggagcattacctggcatggtgtggcaagatagagacgtgtacctgcagggtcccatttgggccaaaattccccacacagatggacactttcacccgtctcctcttatgggcggctttggactcaagaacccgcctcctcaggtcctcatcaaaaacacgcctgttcctgcgaatcctccggcggagttttcagctacaaagtttgcttcattcatcacccaatactccacaggacaagtgagtgtggaaattgaatgggagctgcagaaagaaaacagcaagcgctggaatcccgaagtgcagtacacatccaattatgcaaaatctgccaacgttgattttactgtggacaacaatggactttatactgagcctcgccccattggcacccgttaccttacccgtcccctgtaattacgtgttaatcaataaaccggttaattcgtgtcagttgaactttggtctcatgtcgttattatcttatctggtcaccagatacgtagataagtagcatggcgggttaatcattaactacagcccgggcgtttaaacagcgggcggaggggtggagtcgtgacgtgaattacgtcatagggttagggaggtcctgtattagaggtcacgtgagtgttttgcgacattttgcgacaccatgtggtcacgctgggggggggggcccgagtgagcacgcagggtctccattttgaagcgggaggtttgaacgagcgctggcgcgctcactggccgtcgttttacaacgtcgtgactgggaaaaccctggcgttacccaacttaatcgccttgcagcacatccccctttcgccagctggcgtaatagcgaagaggcccgcaccgatcgcccttcccaacagttgcgcagcctgaatggcgaatgggtaaattgtaaacgttaatattttgttaaaattcgcgttaaatttttgttaaatcagctcattttttaaccaataggccgaaatcggcaaaatcccttataaatcaaaagaatagaccgagatagggttgagtgttgttccagtttggaacaagagtccactattaaagaacgtggactccaacgtcaaagggcgaaaaaccgtctatcagggcgatggcccactacgtgaaccatcaccctaatcaagttttttggggtcgaggtgccgtaaagcactaaatcggaaccctaaagggagcccccgatttagagcttgacggggaaagccggcgaacgtggcgagaaaggaagggaagaaagcgaaaggagcgggcgctagggcgctggcaagtgtagcggtcacgctgcgcgtaaccaccacacccgccgcgcttaatgcgccgctacagggcgcgtggtggcacttttcggggaaatgtgcgcggaacccctatttgtttatttttctaaatacattcaaatatgtatccgctcatgagacaataaccctgataaatgcttcaataatattgaaaaaggaagagtatgagtattcaacatttccgtgtcgcccttattcccttttttgcggcattttgccttcctgtttttgctcacccagaaacgctggtgaaagtaaaagatgctgaagatcagttgggtgcacgagtgggttacatcgaactggatctcaacagcggtaagatccttgagagttttcgccccgaagaacgttttccaatgatgagcacttttaaagttctgctatgtggcgcggtattatcccgtattgacgccgggcaagagcaactcggtcgccgcatacactattctcagaatgacttggttgagtactcaccagtcacagaaaagcatcttacggatggcatgacagtaagagaattatgcagtgctgccataagcatgagtgataacactgcggccaacttacttctgacaacgatcggaggaccgaaggagctaaccgctttttttcacaacatgggggatcatgtaactcgccttgatcgttgggaaccggagctgaatgaagccataccaaacgacgagcgtgacaccacgatgcctgtagcaatggcaacaacgttgcgcaaactattaactggcgaactacttactctagcttcccggcaacaattaatagactggatggaggcggataaagttgcaggaccacttctgcgctcggcccttccggctggctggtttattgctgataaatctggagccggtgagcgtgggtctcgcggtatcattgcagcactggggccagatggtaagccctcccgtatcgtagttatctacacgacgggcagtcaggcaactatggatgaacgaaatagacagatcgctgagataggtgcctcactgattaagcattggtaactgtcagaccaagtttactcatatatactttagattgatttaaaacttcatttttaatttaaaaggatctaggtgaagatcctttttgataatctcatgaccaaaatcccttaacgtgagttttcgttccactgagcgtcagaccccgtagaaaagatcaaaggatcttcttgagatcctttttttctgcgcgtaatctgctgcttgcaaacaaaaaaaccaccgctaccagcggtggtttgtttgccggatcaagagctaccaactctttttccgaaggtaactggcttcagcagagcgcagataccaaatactgtccttctagtgtagccgtagttaggccaccacttcaagaactctgtagcaccgcctacatacctcgctctgctaatcctgttaccagtggctgctgccagtggcgataagtcgtgtcttaccgggttggactcaagacgatagttaccggataaggcgcagcggtcgggctgaacggggggttcgtgcacacagcccagcttggagcgaacgacctacaccgaactgagatacctacagcgtgagcattgagaaagcgccacgcttcccgaagggagaaaggcggacaggtatccggtaagcggcagggtcggaacaggagagcgcacgagggagcttccaggggggaacgcctggtatctttatagtcctgtcgggtttcgccacctctgacttgagcgtcgatttttgtgatgctcgtcaggggggccgagcctatggaaaaacgccagcaacgcggcctttttacggttcctggccttttgctggccttttgctcacatgttctttcctgcgttatcccctgattctgtggataaccgtattaccgcctttgagtgagctgataccgctcgccgcagccgaacgaccgagcgcagcgagtcagtgagcgaggaagcggaagagcgcccaatacgcaaaccgcctctccccgcgcgttggccgattcattaatgcagctggcacgacaggtttcccgactggaaagcgggcagtgagcgcaacgcaattaatgtgagttacctcactcattaggcaccccaggctttacactttatgcttccggctcctatgttgtgtggaattgtgagcggataacaatttcacacaggaaacagctatgaccatgattacgccaa

SEQ ID NO: 6 - DNA, 7328 bp, Adeno-Associated Virus Serotype 1
  source 1..7328: mol_type = genomic DNA
gcgcgccgatatcgttaacgccccgcgccggccgctctagaactagtggatcccccggaagatcagaagttcctattccgaagttcctattctctagaaagtataggaacttctgatctgcgcagccgccatgccggggttttacgagattgtgattaaggtccccagcgaccttgacgggcatctgcccggcatttctgacagctttgtgaactgggtggccgagaaggaatgggagttgccgccagattctgacatggatctgaatctgattgagcaggcacccctgaccgtggccgagaagctgcagcgcgactttctgacggaatggcgccgtgtgagtaaggccccggaggcccttttctttgtgcaatttgagaagggagagagctacttccacatgcacgtgctcgtggaaaccaccggggtgaaatccatggttttgggacgtttcctgagtcagattcgcgaaaaactgattcagagaatttaccgcgggatcgagccgactttgccaaactggttcgcggtcacaaagaccagaaatggcgccggaggcgggaacaaggtggtggatgagtgctacatccccaattacttgctccccaaaacccagcctgagctccagtgggcgtggactaatatggaacagtatttaagcgcctgtttgaatctcacggagcgtaaacggttggtggcgcagcatctgacgcacgtgtcgcagacgcaggagcagaacaaagagaatcagaatcccaattctgatgcgccggtgatcagatcaaaaacttcagccaggtacatggagctggtcgggtggctcgtggacaaggggattacctcggagaagcagtggatccaggaggaccaggcctcatacatctccttcaatgcggcctccaactcgcggtcccaaatcaaggctgccttggacaatgcgggaaagattatgagcctgactaaaaccgcccccgactacctggtgggccagcagcccgtggaggacatttccagcaatcggatttataaaattttggaactaaacgggtacgatccccaatatgcggcttccgtctttctgggatgggccacgaaaaagttcggcaagaggaacaccatctggctgtttgggcctgcaactaccgggaagaccaacatcgcggaggccatagcccacactgtgcccttctacgggtgcgtaaactggaccaatgagaactttcccttcaacgactgtgtcgacaagatggtgatctggtgggaggaggggaagatgaccgccaaggtcgtggagtcggccaaagccattctcggaggaagcaaggtgcgcgtggaccagaaatgcaagtcctcggcccagatagacccgactcccgtgatcgtcacctccaacaccaacatgtgcgccgtgattgacgggaactcaacgaccttcgaacaccagcagccgttgcaagaccggatgttcaaatttgaactcacccgccgtctggatcatgactttgggaaggtcaccaagcaggaagtcaaagactttttccggtgggcaaaggatcacgtggttgaggtggagcatgaattctacgtcaaaaagggtggagccaagaaaagacccgcccccagtgacgcagatataagtgagcccaaacgggtgcgcgagtcagttgcgcagccatcgacgtcagacgcggaagcttcgatcaactacgcagacaggtaccaaaacaaatgttctcgtcacgtgggcatgaatctgatgctgtttccctgcagacaatgcgagagaatgaatcagaattcaaatatctgcttcactcacggacagaaagactgtttagagtgctttcccgtgtcagaatctcaacccgtttctgtcgtcaaaaaggcgtatcagaaactgtgctacattcatcatatcatgggaaaggtgccagacgcttgcactgcctgcgatctggtcaatgtggatttggatgactgcatctttgaacaataaatgatttaaatcaggtatggctgccgatggttatcttccagattggctcgaggacaacctctctgagggcattcgcgagtggtgggacttgaaacctggagccccgaagcccaaagccaaccagcaaaagcaggacgacggccggggtctggtgcttcctggctacaagtacctcggacccttcaacggactcgacaagggggagcccgtcaacgcggcggacgcagcggccctcgagcacgacaaggcctacgaccagcagctcaaagcgggtgacaatccgtaccttcggtataaccacgccgacgccgagtttcaggagcgtctgcaagaagatacgtcttttgggggcaacctcgggcgagcagtcttccaggccaagaagcgggttctcgaacctctcggtctggttgaggaaggcgctaagacggctcctggaaagaaacgtccggtagagcagtcgccacaagagccagactcctcctcgggcatcggcaagacaggccagcagcccgctaaaaagagactcaattttggtcagactggcgactcagagtcagtccccgacccacaacctctcggagaacctccagcaacccccgctgctgtgggacctactacaatggcttcaggcggtggcgcaccaatggcagacaataacgaaggcgccgacggagtgggtaatgcctcaggaaattggcattgcgattccacatggctgggcgacagagtcatcaccaccagcacccgcacctgggccttgcccacctacaataaccacctctacaagcaaatctccagtgcttcaacgggggccagcaacgacaaccactacttcggctacagcaccccctgggggtattttgatttcaacagattccactgccacttttcaccacgtgactggcagcgactcatcaacaacaattggggattccggcccaagagactcaacttcaaactcttcaacatccaagtcaaggaggtcacgacgaatgatggcgtcacaaccatcgctaataaccttaccagcacggttcaagtcttctcggactcggagtaccagcttccgtacgtcctcggctctgcgcaccagggctgcctccctccgttcccggcggacgtgttcatgattccgcaatacggctacctgacgctcaacaatggcagccaagccgtgggacgttcatccttttactgcctggaatatttcccttctcagatgctgagaacgggcaacaactttaccttcagctacacctttgaggaagtgcctttccacagcagctacgcgcacagccagagcctggaccggctgatgaatcctctcatcgaccaatacctgtattacctgaacagaactcaaaatcagtccggaagtgcccaaaacaaggacttgctgtttagccgtgggtctccagctggcatgtctgttcagcccaaaaactggctacctggaccctgttatcggcagcagcgcgtttctaaaacaaaaacagacaacaacaacagcaattttacctggactggtgcttcaaaatataacctcaatgggcgtgaatccatcatcaaccctggcactgctatggcctcacacaaagacgacgaagacaagttctttcccatgagcggtgtcatgatttttggaaaagagagcgccggagcttcaaacactgcattggacaatgtcatgattacagacgaagaggaaattaaagccactaaccctgtggccaccgaaagatttgggaccgtggcagtcaatttccagagcagcagcacagaccctgcgaccggagatgtgcatgctatgggagcattacctggcatggtgtggcaagatagagacgtgtacctgcagggtcccatttgggccaaaattccccacacagatggacactttcacccgtctcctcttatgggcggctttggactcaagaacccgcctcctcagatcctcatcaaaaacacgcctgttcctgcgaatcctccggcggagttttcagctacaaagtttgcttcattcatcacccaatactccacaggacaagtgagtgtggaaattgaatgggagctgcagaaagaaaacagcaagcgctggaatcccgaagtgcagtacacatccaattatgcaaaatctgccaacgttgattttactgtggacaacaatggactttatactgagcctcgccccattggcacccgttaccttacccgtcccctgtaattacgtgttaatcaataaaccggttaattcgtgtcagttgaactttggtctcatgtcgttattatcttatctggtcaccagatacgtagataagtagcatggcgggttaatcattaactacagcccgggcgtttaaacagcgggcggaggggtggagtcgtgacgtgaattacgtcatagggttagggaggtcctgtattagaggtcacgtgagtgttttgcgacattttgcgacaccatgtggtcacgctgggggggggggcccgagtgagcacgcagggtctccattttgaagcgggaggtttgaacgagcgctggcgcgctcactggccgtcgttttacaacgtcgtgactgggaaaaccctggcgttacccaacttaatcgccttgcagcacatccccctttcgccagctggcgtaatagcgaagaggcccgcaccgatcgcccttcccaacagttgcgcagcctgaatggcgaatgggtaaattgtaaacgttaatattttgttaaaattcgcgttaaatttttgttaaatcagctcattttttaaccaataggccgaaatcggcaaaatcccttataaatcaaaagaatagaccgagatagggttgagtgttgttccagtttggaacaagagtccactattaaagaacgtggactccaacgtcaaagggcgaaaaaccgtctatcagggcgatggcccactacgtgaaccatcaccctaatcaagttttttggggtcgaggtgccgtaaagcactaaatcggaaccctaaagggagcccccgatttagagcttgacggggaaagccggcgaacgtggcgagaaaggaagggaagaaagcgaaaggagcgggcgctagggcgctggcaagtgtagcggtcacgctgcgcgtaaccaccacacccgccgcgcttaatgcgccgctacagggcgcgtggtggcacttttcggggaaatgtgcgcggaacccctatttgtttatttttctaaatacattcaaatatgtatccgctcatgagacaataaccctgataaatgcttcaataatattgaaaaaggaagagtatgagtattcaacatttccgtgtcgcccttattcccttttttgcggcattttgccttcctgtttttgctcacccagaaacgctggtgaaagtaaaagatgctgaagatcagttgggtgcacgagtgggttacatcgaactggatctcaacagcggtaagatccttgagagttttcgccccgaagaacgttttccaatgatgagcacttttaaagttctgctatgtggcgcggtattatcccgtattgacgccgggcaagagcaactcggtcgccgcatacactattctcagaatgacttggttgagtactcaccagtcacagaaaagcatcttacggatggcatgacagtaagagaattatgcagtgctgccataagcatgagtgataacactgcggccaacttacttctgacaacgatcggaggaccgaaggagctaaccgctttttttcacaacatgggggatcatgtaactcgccttgatcgttgggaaccggagctgaatgaagccataccaaacgacgagcgtgacaccacgatgcctgtagcaatggcaacaacgttgcgcaaactattaactggcgaactacttactctagcttcccggcaacaattaatagactggatggaggcggataaagttgcaggaccacttctgcgctcggcccttccggctggctggtttattgctgataaatctggagccggtgagcgtgggtctcgcggtatcattgcagcactggggccagatggtaagccctcccgtatcgtagttatctacacgacgggcagtcaggcaactatggatgaacgaaatagacagatcgctgagataggtgcctcactgattaagcattggtaactgtcagaccaagtttactcatatatactttagattgatttaaaacttcatttttaatttaaaaggatctaggtgaagatcctttttgataatctcatgaccaaaatcccttaacgtgagttttcgttccactgagcgtcagaccccgtagaaaagatcaaaggatcttcttgagatcctttttttctgcgcgtaatctgctgcttgcaaacaaaaaaaccaccgctaccagcggtggtttgtttgccggatcaagagctaccaactctttttccgaaggtaactggcttcagcagagcgcagataccaaatactgtccttctagtgtagccgtagttaggccaccacttcaagaactctgtagcaccgcctacatacctcgctctgctaatcctgttaccagtggctgctgccagtggcgataagtcgtgtcttaccgggttggactcaagacgatagttaccggataaggcgcagcggtcgggctgaacggggggttcgtgcacacagcccagcttggagcgaacgacctacaccgaactgagatacctacagcgtgagcattgagaaagcgccacgcttcccgaagggagaaaggcggacaggtatccggtaagcggcagggtcggaacaggagagcgcacgagggagcttccaggggggaacgcctggtatctttatagtcctgtcgggtttcgccacctctgacttgagcgtcgatttttgtgatgctcgtcaggggggccgagcctatggaaaaacgccagcaacgcggcctttttacggttcctggccttttgctggccttttgctcacatgttctttcctgcgttatcccctgattctgtggataaccgtattaccgcctttgagtgagctgataccgctcgccgcagccgaacgaccgagcgcagcgagtcagtgagcgaggaagcggaagagcgcccaatacgcaaaccgcctctccccgcgcgttggccgattcattaatgcagctggcacgacaggtttcccgactggaaagcgggcagtgagcgcaacgcaattaatgtgagttacctcactcattaggcaccccaggctttacactttatgcttccggctcctatgttgtgtggaattgtgagcggataacaatttcacacaggaaacagctatgaccatgattacgccaa

SEQ ID NO: 7 - DNA, 22 bp, Artificial Sequence
  source 1..22: mol_type = unassigned DNA
gcggaagcttcgatcaactacg

SEQ ID NO: 8 - DNA, 23 bp, Artificial Sequence
  source 1..23: mol_type = unassigned DNA
cgcagagaccaaagttcaactga

SEQ ID NO: 9 - DNA, 22 bp, Artificial Sequence
  source 1..22: mol_type = unassigned DNA
gcggaagcttcgatcaactacg

SEQ ID NO: 10 - DNA, 23 bp, Artificial Sequence
  source 1..23: mol_type = unassigned DNA
cgcagagaccaaagttcaactga

SEQ ID NO: 11 - DNA, 21 bp, Artificial Sequence
  source 1..21: mol_type = unassigned DNA
atggtgatgcggttttggcag

SEQ ID NO: 12 - DNA, 24 bp, Artificial Sequence
  source 1..24: mol_type = unassigned DNA
ggcggagttgttacgacattttgg